European Patent Application EP 4 148 119 A1, published March 15, 2023. Title: Novel Lactic Acid Bacteria with Excellent Immune function enhancing effect and Food Composition Containing the Same and Health Functional Food Composition Containing the Same and Probiotics comprising the Same. Applicant: GREEN CROSS WellBeing Corporation. The sequence listing filed with the application follows.

SEQUENCE LISTING (1 sequence)

SEQ ID NO: 1 - RNA, 1481 nt, Artificial Sequence
  artificial sequence
ctcaggacgaacgctggcggcgtgcctaatacatgcaagttgagcgctgaaggttggtacttgtaccaactggatgagcagcgaacgggtgagtaacgcgtggggaatctgcctttgagcgggggacaactttggaaacgaatgctaataccgcataaaaactttaaacacaagttttaagtttgaaagatgcaattgcatcactcaaagatgatcccgcgttgtattagctagttggtgaggtaaaggctcaccaaggcgatgatacatagccgacctgagagggtgatcggccacattgggactgagacacggcccaaactcctacgggaggcagcagtagggaatcttcggcaatggacgaaagtctgaccgagcaacgccgcgtgagtgaagaaggttttcggatcgtaaaactctgttggtagagaagaacgttggtgagagtggaaagctcatcaagtgacggtaactacccagaaagggacggctaactacgtgccagcagccgcggtaatacgtaggtcccgagcgttgtccggatttattgggcgtaaagcgagcgcaggtggtttattaagtctggtgtaaaaggcagtggctcaaccattgtatgcattggaaactggtagacttgagtgcaggagaggagagtggaattccatgtgtagcggtgaaatgcgtagatatatggaggaacaccggtggcgaaagcggctctctggcctgtaactgacactgaggctcgaaagcgtggggagcaaacaggattagataccctggtagtccacgccgtaaacgatgagtgctagatgtagggagctataagttctctgtatcgcagctaacgcaataagcactccgcctggggagtacgaccgcaaggttgaaactcaaaggaattgacgggggcccgcacaagcggtggagcatgtggtttaattcgaagcaacgcgaagaaccttaccaggtcttgacatactcgtgctattcctagagataggaagttccttcgggacacgggatacaggtggtgcatggttgtcgtcagctcgtgtcgtgagatgttgggttaagtcccgcaacgagcgcaacccctattgttagttgccatcattaagttgggcactctaacgagactgccggtgataaaccggaggaaggtggggatgacgtcaaatcatcatgccccttatgacctgggctacacacgtgctacaatggatggtacaacgagtcgcgagacagtgatgtttagctaatctcttaaaaccattctcagttcggattgtaggctgcaactcgcctacatgaagtcggaatcgctagtaatcgcggatcagcacgccgcggtgaatacgttcccgggccttgtacacaccgcccgtcacaccacgggagttgggagtacccgaagtaggttgcctaaccgcaaggagggcgcttcctaaggtaagaccgatgactggggtgaagtcgta